European Patent Application EP 4 261 227 A1, published October 18, 2023. Title: 一种鼠抗OXA-48型碳青霉烯酶杂交瘤细胞株，单克隆抗体及应用. Applicant: 天津一瑞生物科技股份有限公司. The sequence listing filed with the application follows.

SEQUENCE LISTING (20 sequences)

SEQ ID NO: 1 - protein, 11 aa, Artificial sequence
RASKSISKYLA

SEQ ID NO: 2 - protein, 7 aa, Artificial sequence
SGSTFQS

SEQ ID NO: 3 - protein, 10 aa, Artificial sequence
QQHNEYPYVT

SEQ ID NO: 4 - protein, 10 aa, Artificial sequence
GFTFSTYAMS

SEQ ID NO: 5 - protein, 17 aa, Artificial sequence
TISSGGSYTSYPDSVKG

SEQ ID NO: 6 - protein, 8 aa, Artificial sequence
RPEYAMDY

SEQ ID NO: 7 - protein, 114 aa, Artificial sequence
DWIQLVQHQPVSSYLAASPGETVTINCRASKSISKYLAWYQEKPGKTNKLLIYSGSTFQSGFPSGFSGSGSGTDFTLTVSSLEPEDFAIYYCQQHNEYPYVTFGGGTKLEIKRA

SEQ ID NO: 8 - DNA, 342 bp, Artificial sequence
  source 1..342: mol_type = other DNA
gattggatacagttggtgcagcatcagcccgtttcatcttatcttgctgcatctcctggagaaaccgttactattaattgcagggcaagtaagagcattagcaagtatttagcctggtatcaagagaaacctgggaaaactaataagcttcttatctactctggttccactttccaatctggatttccatcagggttcagtggcagtggatctggtacagatttcactctcaccgtcagtagcctggagcctgaagactttgcaatctattactgtcaacagcataatgagtacccgtacgtcacgttcggaggggggaccaagctggagataaaacgggct

SEQ ID NO: 9 - protein, 120 aa, Artificial sequence
QCEVMLVESGGGLVKPGGSLKLSCAASGFTFSTYAMSWVRLTPEKRLEWVATISSGGSYTSYPDSVKGRFTISRDNAKNTLYLQMSSLRSEDTAMYYCARRPEYAMDYWGQGTSVTVSSA

SEQ ID NO: 10 - DNA, 360 bp, Artificial sequence
  source 1..360: mol_type = other DNA
cagtgtgaagtgatgctggtggagtctgggggaggcttagtgaagcctggagggtccctgaaactctcctgtgcagcctctggattcactttcagtacctatgccatgtcttgggttcgcctgactccggagaagaggctggagtgggtcgcaaccattagtagtggtggtagttacacctcctatccagacagtgtgaaggggcgcttcaccatctccagagacaatgccaagaacaccctgtacctgcaaatgagcagtctgaggtctgaggacacggccatgtattactgtgcacgacgacccgaatatgctatggactactggggtcaaggaacctcagtcaccgtctcctcagcc

SEQ ID NO: 11 - protein, 15 aa, Artificial sequence
RASKSVSTSGYSYMH

SEQ ID NO: 12 - protein, 7 aa, Artificial sequence
LVSNLES

SEQ ID NO: 13 - protein, 8 aa, Artificial sequence
QHIRELYT

SEQ ID NO: 14 - protein, 10 aa, Artificial sequence
GYTFTDYVIS

SEQ ID NO: 15 - protein, 17 aa, Artificial sequence
EIYPGSDTTYHNEKFKG

SEQ ID NO: 16 - protein, 11 aa, Artificial sequence
DYGSNYGWFAY

SEQ ID NO: 17 - protein, 110 aa, Artificial sequence
DIVLTQSPASLAVSLGQRATISYRASKSVSTSGYSYMHWNQQKPGQPPRLLIYLVSNLESGVPARFSGSGSGTDFTLNIHPVEEEDAATYYCQHIRELYTFGGGTKLEIK

SEQ ID NO: 18 - DNA, 330 bp, Artificial sequence
  source 1..330: mol_type = other DNA
gacattgtgctgacacagtctcctgcttccttagctgtatctctggggcagagggccaccatctcatacagggccagcaaaagtgtcagtacatctggctatagttatatgcactggaaccaacagaaaccaggacagccacccagactcctcatctatcttgtatccaacctagaatctggggtccctgccaggttcagtggcagtgggtctgggacagacttcaccctcaacatccatcctgtggaggaggaggatgctgcaacctattactgtcagcacattagggagctttacacgttcggaggggggaccaagctggaaataaaa

SEQ ID NO: 19 - protein, 120 aa, Artificial sequence
EVKLQQSGPELVKPGASVKMSCMASGYTFTDYVISWVKQRNGQGLEWIGEIYPGSDTTYHNEKFKGKATLTADISSNTVYMQLSSLTFEDSAVYFCARDYGSNYGWFAYWGQGTLVTVSA

SEQ ID NO: 20 - DNA, 360 bp, Artificial sequence
  source 1..360: mol_type = other DNA
gaggtgaagctgcagcagtctggacctgagttggtgaagcctggggcttcagtgaagatgtcctgcatggcttctggatacacattcactgactatgttataagttgggtgaagcagagaaatggacagggccttgagtggattggagagatttatcctggaagtgataccacttaccacaatgagaaattcaagggcaaggccacactgactgcagacatatcctccaacacagtctacatgcagctcagtagtctgacatttgaggattctgcggtctatttctgtgcaagagactacggtagtaactacggctggtttgcttactggggccaagggactctggtcactgtctctgca